European Patent Application EP 4 803 532 A1, published September 9, 2026. Title: 非洲猪瘟病毒CD2v蛋白的免疫原性组合物及其应用. Applicant: 广东蓝玉生物科技有限公司. The sequence listing filed with the application follows.

SEQUENCE LISTING (21 sequences)

SEQ ID NO: 1 - protein, 360 aa, synthetic construct
MIILIFLIFSNIVLSIDYWVSFNKTIILDSNITNDNNDINGVSWNFFNNSFNTLATCGKAGNFCECSNYSTSIYNITNNCSLTIFPHNDVFDTTYQVVWNQIINYTIKLLTPATPPNITYNCTNFLITCKKNNGTNTNIYLNINDTFVKYTNESILEYNWNNSNINNFTATCIINNTISTSNETTLINCTYLTLSSNYFYTFFKLYYIPLSIIIGITISILLISIITFLSLRKRKKHVEEIESPPPESNEEEQCQHDDTTSIHEPSPREPLLPKPYSRYQYNTPIYYMRPSTQPLNPFPLPKPCPPPKPCPPPKPCPPPKPCPSAESYSPPKPLPSIPLLPNIPPLSTQNISLIHVDRII

SEQ ID NO: 2 - protein, 91 aa, synthetic construct
SNIVLSIDYWVSFNKTIILDSNITNDNNDINGVSWNFFNNSFNTLATCGKAGNFCECSNYSTSIYNITNNCSLTIFPHNDVFDTTYQVVWN

SEQ ID NO: 3 - protein, 97 aa, synthetic construct
SNIVLSIDYWVSFNKTIILDSNITNDNNDINGVSWNFFNNSFNTLATCGKAGNFCECSNYSTSIYNITNNCSLTIFPHNDVFDTTYQVVWNQIINYT

SEQ ID NO: 4 - protein, 100 aa, synthetic construct
SNIVLSIDYWVSFNKTIILDSNITNDNNDINGVSWNFFNNSFNTLATCGKAGNFCECSNYSTSIYNITNNCSLTIFPHNDVFDTTYQVVWNQIINYTIKL

SEQ ID NO: 5 - protein, 83 aa, synthetic construct
YWVSFNKTIILDSNITNDNNDINGVSWNFFNNSFNTLATCGKAGNFCECSNYSTSIYNITNNCSLTIFPHNDVFDTTYQVVWN

SEQ ID NO: 6 - protein, 89 aa, synthetic construct
YWVSFNKTIILDSNITNDNNDINGVSWNFFNNSFNTLATCGKAGNFCECSNYSTSIYNITNNCSLTIFPHNDVFDTTYQVVWNQIINYT

SEQ ID NO: 7 - protein, 90 aa, synthetic construct
YWVSFNKTIILDSNITNDNNDINGVSWNFFNNSFNTLATCGKAGNFCECSNYSTSIYNITNNCSLTIFPHNDVFDTTYQVVWNQIINYTI

SEQ ID NO: 8 - protein, 92 aa, synthetic construct
YWVSFNKTIILDSNITNDNNDINGVSWNFFNNSFNTLATCGKAGNFCECSNYSTSIYNITNNCSLTIFPHNDVFDTTYQVVWNQIINYTIKL

SEQ ID NO: 9 - protein, 97 aa, synthetic construct
KLLTPATPPNITYNCTNFLITCKKNNGTNTNIYLNINDTFVKYTNESILEYNWNNSNINNFTATCIINNTISTSNETTLINCTYLTLSSNYFYTFFK

SEQ ID NO: 10 - protein, 94 aa, synthetic construct
TPATPPNITYNCTNFLITCKKNNGTNTNIYLNINDTFVKYTNESILEYNWNNSNINNFTATCIINNTISTSNETTLINCTYLTLSSNYFYTFFK

SEQ ID NO: 11 - protein, 91 aa, synthetic construct
TPPNITYNCTNFLITCKKNNGTNTNIYLNINDTFVKYTNESILEYNWNNSNINNFTATCIINNTISTSNETTLINCTYLTLSSNYFYTFFK

SEQ ID NO: 12 - protein, 88 aa, synthetic construct
NITYNCTNFLITCKKNNGTNTNIYLNINDTFVKYTNESILEYNWNNSNINNFTATCIINNTISTSNETTLINCTYLTLSSNYFYTFFK

SEQ ID NO: 13 - protein, 205 aa, synthetic construct
MEELFKKHKIVAVLRANSVEEAIEKAVAVFAGGVHLIEITFTVPDADTVIKALSVLKEKGAIIGAGTVTSVEQCRKAVESGAEFIVSPHLDEEISQFCKEKGVFYMPGVMTPTELVKAMKLGHTILKLFPGEVVGPQFVKAMKGPFPNVKFVPTGGVNLDNVCEWFKAGVLAVGVGSALVKGTPDEVREKAKAFVEKIRGCTELE

SEQ ID NO: 14 - protein, 161 aa, synthetic construct
MNQHSHKDHETVRIAVVRARWHAEIVDACVSAFEAAMRDIGGDRFAVDVFDVPGAYEIPLHARTLAETGRYGAVLGTAFVVNGGIYRHEFVASAVINGMMNVQLNTGVPVLSAVLTPHNYDKSKAHTLLFLALFAVKGMEAARACVEILAAREKIAAGSLE

SEQ ID NO: 15 - protein, 138 aa, synthetic construct
MGMKEKFVLIITHGDFGKGLLSGAEVIIGKQENVHTVGLNLGDNIEKVAKEVMRIIIAKLAEDKEIIIVVDLFGGSPFNIALEMMKTFDVKVITGINMPMLVELLTSINVYDTTELLENISKIGKDGIKVIEKSSLKM

SEQ ID NO: 16 - protein, 158 aa, synthetic construct
MILSAEQSFTLRHPHGQAAALAFVREPAAALAGVQRLRGLDSDGEQVWGELLVRVPLLGEVDLPFRSEIVRTPQGAELRPLTLTGERAWVAVSGQATAAEGGEMAFAFQFQAHLATPEAEGEGGAAFEVMVQAAAGVTLLLVAMALPQGLAAGLPALE

SEQ ID NO: 17 - protein, 154 aa, synthetic construct
MQIYEGKLTAEGLRFGIVASRFNHALVDRLVEGAIDCIVRHGGREEDITLVRVPGSWEIPVAAGELARKEDIDAVIAIGVLIRGATPHFDYIASEVSKGLANLALELRKPITFGVITADTLEQAIERAGTKHGNKGWEAALSAIEMANLFKSLR

SEQ ID NO: 18 - protein, 242 aa, synthetic construct
AAAKPATTEGEFPETREKMSGIRRAIAKAMVHSKHTAPHVTLMDEADVTKLVAHRKKFKAIAAEKGIKLTFLPYVVKALVSALREYPVLNTAIDDETEEIIQKHYYNIGIAADTDRGLLVPVIKHADRKPIFALAQEINELAEKARDGKLTPGEMKGASCTITNIGSAGGQWFTPVINHPEVAILGIGRIAEKPIVRDGEIVAAPMLALSLSFDHRMIDGATAQKALNHIKRLLSDPELLLM

SEQ ID NO: 19 - protein, 205 aa, synthetic construct
MKMEELFKKHKIVAVLRANSVEEAKKKALAVFLGGVHLIEITFTVPDADTVIKELSFLKEMGAIIGAGTVTSVEQCRKAVESGAEFIVSPHLDEEISQFCKEKGVFYMPGVMTPTELVKAMKLGHTILKLFPGEVVGPQFVKAMKGPFPNVKFVPTGGVNLDNVCEWFKAGVLAVGVGSALVKGTPVEVAEKAKAFVEKIRGCTE

SEQ ID NO: 20 - protein, 6 aa, synthetic construct
HHHHHH

SEQ ID NO: 21 - protein, 10 aa, synthetic construct
GGGGSGGGGS